European Patent Specification EP 3 762 333 B1, published March 1, 2023. Title: Composite material comprising DNA hydrogel and silica nanoparticles. Applicant: KIT. The sequence listing filed with the application follows.

SEQUENCE LISTING (17 sequences)

SEQ ID NO: 1 - DNA, 58 bp, Artificial Sequence
  oligonucleotide for preparing DNA hairpins for the linear HCR process
gatcgcgatcctggctcctgtgattgtgctctagacatcgctagagcacaatcacagg

SEQ ID NO: 2 - DNA, 52 bp, Artificial Sequence
  oligonucleotide for preparing DNA hairpins for the linear HCR process
ctagagcacaatcacaggagccagttttcctgtgattgtgctctagcgatgt

SEQ ID NO: 3 - DNA, 44 bp, Artificial Sequence
  initiator for HCR process
  amino-modified (1)..(1)
ttttttttttttttttttttcatctcagtctaggattcggcgtg

SEQ ID NO: 4 - DNA, 50 bp, Artificial Sequence
  oligonucleotide for preparing DNA hairpins for the linear HCR process
agtctaggattcggcgtgacgactttcacgccgaatcctagactgagatg

SEQ ID NO: 5 - DNA, 76 bp, Artificial Sequence
  oligonucleotide for preparing DNA hairpins for the linear HCR process
acatcgctagagcacaatcacaggttagtcgtcacgccgaatcctagactttcatctcagtctaggattcggcgtg

SEQ ID NO: 6 - DNA, 24 bp, Artificial Sequence
  initiator for HCR process
acatcgctagagcacaatcacagg

SEQ ID NO: 7 - DNA, 52 bp, Artificial Sequence
  primer for SiNP modification
  amino-modified (1)..(1)
tttttttttttttctaactgctgcgccgccgggaaaatactgtacggttaga

SEQ ID NO: 8 - DNA, 80 bp, Artificial Sequence
  primer for CNT modification
tttttttttttttttttttttttttttttttttttttttttctaactgctgcgccgccgggaaaatactgtacggttaga

SEQ ID NO: 9 - DNA, 41 bp, Artificial Sequence
  aptamer which specifically binds to the PTK7 receptor
atctaactgctgcgccgccgggaaaatactgtacggttaga

SEQ ID NO: 10 - DNA, 98 bp, Artificial Sequence
  template for RCA
  phosphorylated (1)..(1)
ttcccggcggcgcagcagttagatgctgctgcagcgatacgcgtatcgctatgggtaaccgtacggttacccgcagcagcatctaaccgtacagtatt

SEQ ID NO: 11 - DNA, 98 bp, Artificial Sequence
  template for simultaneous RCA and HCR
  phosphorylated (1)..(1)
ttcccggcggcgcagcagttagatgctgctgcagcgaacatcgctagagcacaatcacaggtacgatatgccgcagcagcatctaaccgtacagtatt

SEQ ID NO: 12 - DNA, 52 bp, Artificial Sequence
  primer for PCR on mKate-producing plasmid
cgtacgatatgccatagcgatacgcggcggtttgcgtattgggcgctcttcc

SEQ ID NO: 13 - DNA, 20 bp, Artificial Sequence
  primer for PCR on mKate-producing plasmid
ctctccccgcgcgttggccg

SEQ ID NO: 14 - DNA, 6210 bp, Artificial Sequence
  plasmid for PCR
gacggatcgggagatctcccgatcccctatggtgcactctcagtacaatctgctctgatgccgcatagttaagccagtatctgctccctgcttgtgtgttggaggtcgctgagtagtgcgcgagcaaaatttaagctacaacaaggcaaggcttgaccgacaattgcatgaagaatctgcttagggttaggcgttttgcgctgcttcgcgatgtacgggccagatatacgcgttgacattgattattgactagttattaatagtaatcaattacggggtcattagttcatagcccatatatggagttccgcgttacataacttacggtaaatggcccgcctggctgaccgcccaacgacccccgcccattgacgtcaataatgacgtatgttcccatagtaacgccaatagggactttccattgacgtcaatgggtggagtatttacggtaaactgcccacttggcagtacatcaagtgtatcatatgccaagtacgccccctattgacgtcaatacggtaaatggcccgcctggcattatgcccagtacatgaccttatgggactttcctacttggcagtacatctacgtattagtcatcgctattaccatggtgatgcggttttggcagtacatcaatgggcgtggatagcggtttgactcacggggatttccaagtctccaccccattgacgtcaatgggagtttgttttggcaccaaaatcacgggactttccaaaatgtcgtaacaactccgccccattgacgcaaatgggcggtaggcgtgtacggtgggaggtctatataagcagagctctctggctaactagagaacccactgcttactggcttatcgaaattaatacgactcactatagggagacccaagctggctagttaagctatcaacaagtttgtacaaaaagcaggctctaaggaggatagaaccatggtgtctaagggcgaagagctgattaaggagaacatgcacatgaagctgtacatggagggcaccgtgaacaaccaccacttcaagtgcacatccgagggcgaaggcaagccctacgagggcacccagaccatgagaatcaaggtggtcgagggcggccctctccccttcgccttcgacatcctggctaccagcttcatgtacggcagcaaaaccttcatcaaccacacccaggcatccccgacttctttaagcagtccttccctgagggcttcacatgggagagagtcaccacatacgaagacgggggcgtgctgaccgctacccaggacaccagcctccaggacggctgcctctctacaacgtcaagatcagaggggtgaacttcccatccaacggccctgtgatgcagaagaaaacactcggctgggaggcctccaccgagatgctgtaccccgctgacggcggcctggaaggcagaagcgacatggccctgaagctcgtgggcgggggccacctgatctgcaacttgaagaccacatacagatccaagaaacccgctaagaacctcaagatgcccggcgtctactatgtggacagaagactggaaagaatcaaggaggccgacaaagagacctacgtcgagcagcacgaggtggctgtggccagatactgcgacctccctagcaaactggggcacaaacttaattacccagctttcttgtacaaagtggttgatctagagggcccgcggttcgaaggtaagcctatccctaaccctctcctcggtctcgattctacgcgtaccggtcatcatcaccatcaccattgagtttaaacccgctgatcagcctcgactgtgccttctagttgccagccatctgttgtttgcccctcccccgtgccttccttgaccctggaaggtgccactcccactgtccttcctaataaaatgaggaaattgcatcgcattgtctgagtaggtgtcattctattctggggggtggggtggggcaggacagcaagggggaggattgggaagacaatagcaggcatgctggggatgcggtgggctctatggcttctgaggcggaaagaaccagctggggctctagggggtatccccacgcgccctgtagcggcgcattaagcgcggcgggtgtggtggttacgcgcagcgtgaccgctacacttgccagcgccctagcgcccgctcctttcgctttcttcccttcctttctcgccacgttcgccggctttccccgtcaagctctaaatcgggggctccctttagggttccgatttagtgctttacggcacctcgaccccaaaaaacttgattagggtgatggttcacgtagtgggccatcgccctgatagacggtttttcgccctttgacgttggagtccacgttctttaatagtggactcttgttccaaactggaacaacactcaaccctatctcggtctattcttttgatttataagggattttgccgatttcggcctattggttaaaaaatgagctgatttaacaaaaatttaacgcgaattaattctgtggaatgtgtgtcagttagggtgtggaaagtccccaggctccccagcaggcagaagtatgcaaagcatgcatctcaattagtcagcaaccaggtgtggaaagtccccaggctccccagcaggcagaagtatgcaaagcatgcatctcaattagtcagcaaccatagtcccgcccctaactccgcccatcccgcccctaactccgcccagttccgcccattctccgccccatggctgactaattttttttatttatgcagaggccgaggccgcctctgcctctgagctattccagaagtagtgaggaggcttttttggaggcctaggcttttgcaaaaagctcccgggagcttgtatatccattttcggatctgatcaagagacaggatgaggatcgtttcgcatgattgaacaagatggattgcacgcaggttctccggccgcttgggtggagaggctattcggctatgactgggcacaacagacaatcggctgctctgatgccgccgtgttccggctgtcagcgcaggggcgcccggttctttttgtcaagaccgacctgtccggtgccctgaatgaactgcaggacgaggcagcgcggctatcgtggctggccacgacgggcgttccttgcgcagctgtgctcgacgttgtcactgaagcgggaagggactggctgctattgggcgaagtgccggggcaggatctcctgtcatctcaccttgctcctgccgagaaagtatccatcatggctgatgcaatgcggcggctgcatacgcttgatccggctacctgcccattcgaccaccaagcgaaacatcgcatcgagcgagcacgtactcggatggaagccggtcttgtcgatcaggatgatctggacgaagagcatcaggggctcgcgccagccgaactgttcgccaggctcaaggcgcgcatgcccgacggcgaggatctcgtcgtgacccatggcgatgcctgcttgccgaatatcatggtggaaaatggccgcttttctggattcatcgactgtggccggctgggtgtggcggaccgctatcaggacatagcgttggctacccgtgatattgctgaagagcttggcggcgaatgggctgaccgcttcctcgtgctttacggtatcgccgctcccgattcgcagcgcatcgccttctatcgccttcttgacgagttcttctgagcgggctctggggttcgcgaaatgaccgaccaagcgacgcccaacctgccatcacgagatttcgattccaccgccgccttctatgaaaggttgggcttcggaatcgttttccgggacgccggctggatgatcctccagcgcggggatctcatgctggagttcttcgcccaccccaacttgtttattgcagcttataatggttacaaataaagcaatagcatcacaaatttcacaaataaagcatttttttcactgcattctagttgtggtttgtccaaactcatcaatgtatcttatcatgtctgtataccgtcgacctctagctagagcttggcgtaatcatggtcatagctgtttcctgtgtgaaattgttatccgctcacaattccacacaacatacgagccggaagcataaagtgtaaagcctggggtgcctaatgagtgagctaactcacattaattgcgttgcgctcactgcccgctttccagtcgggaaacctgtcgtgccagctgcattaatgaatcggccaacgcgcggggagaggcggtttgcgtattgggcgctcttccgcttcctcgctcactgactcgctgcgctcggtcgttcggctgcggcgagcggtatcagctcactcaaaggcggtaatacggttatccacagaatcaggggataacgcaggaaagaacatgtgagcaaaaggccagcaaaaggccaggaaccgtaaaaaggccgcgttgctggcgtttttccataggctccgcccccctgacgagcatcacaaaaatcgacgctcaagtcagaggtggcgaaacccgacaggactataaagataccaggcgtttccccctggaagctccctcgtgcgctctcctgttccgaccctgccgcttaccggatacctgtccgcctttctcccttcgggaagcgtggcgctttctcatagctcacgctgtaggtatctcagttcggtgtaggtcgttcgctccaagctgggctgtgtgcacgaaccccccgttcagcccgaccgctgcgccttatccggtaactatcgtcttgagtccaacccggtaagacacgacttatcgccactggcagcagccactggtaacaggattagcagagcgaggtatgtaggcggtgctacagagttcttgaagtggtggcctaactacggctacactagaagaacagtatttggtatctgcgctctgctgaagccagttaccttcggaaaaagagttggtagctcttgatccggcaaacaaaccaccgctggtagcggtggtttttttgtttgcaagcagcagattacgcgcagaaaaaaaggatctcaagaagatcctttgatcttttctacggggtctgacgctcagtggaacgaaaactcacgttaagggattttggtcatgagattatcaaaaaggatcttcacctagatccttttaaattaaaaatgaagttttaaatcaatctaaagtatatatgagtaaacttggtctgacagttaccaatgcttaatcagtgaggcacctatctcagcgatctgtctatttcgttcatccatagttgcctgactccccgtcgtgtagataactacgatacgggagggcttaccatctggccccagtgctgcaatgataccgcgagacccacgctcaccggctccagatttatcagcaataaaccagccagccggaagggccgagcgcagaagtggtcctgcaactttatccgcctccatccagtctattaattgttgccgggaagctagagtaagtagttcgccagttaatagtttgcgcaacgttgttgccattgctacaggcatcgtggtgtcacgctcgtcgtttggtatggcttcattcagctccggttcccaacgatcaaggcgagttacatgatcccccatgttgtgcaaaaaagcggttagctccttcggtcctccgatcgttgtcagaagtaagttggccgcagtgttatcactcatggttatggcagcactgcataattctcttactgtcatgccatccgtaagatgcttttctgtgactggtgagtactcaaccaagtcattctgagaatagtgtatgcggcgaccgagttgctcttgcccggcgtcaatacgggataataccgcgccacatagcagaactttaaaagtgctcatcattggaaaacgttcttcggggcgaaaactctcaaggatcttaccgctgttgagatccagttcgatgtaacccactcgtgcacccaactgatcttcagcatcttttactttcaccagcgtttctgggtgagcaaaaacaggaaggcaaaatgccgcaaaaaagggaataagggcgacacggaaatgttgaatactcatactcttcctttttcaatattattgaagcatttatcagggttattgtctcatgagcggatacatatttgaatgtatttagaaaaataaacaaataggggttccgcgcacatttccccgaaaagtgccacctgacgtc

SEQ ID NO: 15 - DNA, 40 bp, Artificial Sequence
  primer for PCR for PCR on eGFP-producing plasmid
cgcggcggcccttttatgacggacaggtatccggtaagcg

SEQ ID NO: 16 - DNA, 20 bp, Artificial Sequence
  primer for PCR for PCR on eGFP-producing plasmid
ggcggtgctacagagttctt

SEQ ID NO: 17 - DNA, 6130 bp, Artificial Sequence
  plasmid for PCR
gctgagttggctgctgccaccgctgagcaataactagcataaccccttggggcctctaaacgggtcttgaggggttttttgctgaaaggaggaactatatccggattggcgaatgggacgcgccctgtagcggcgcattaagcgcggcgggtgtggtggttacgcgcagcgtgaccgctacacttgccagcgccctagcgcccgctcctttcgctttcttcccttcctttctcgccacgttcgccggctttccccgtcaagctctaaatcgggggctccctttagggttccgatttagtgctttacggcacctcgaccccaaaaaacttgattagggtgatggttcacgtagtgggccatcgccctgatagacggtttttcgccctttgacgttggagtccacgttctttaatagtggactcttgttccaaactggaacaacactcaaccctatctcggtctattcttttgatttataagggattttgccgatttcggcctattggttaaaaaatgagctgatttaacaaaaatttaacgcgaattttaacaaaatattaacgtttacaatttcaggtggcacttttcggggaaatgtgcgcggaacccctatttgtttatttttctaaatacattcaaatatgtatccgctcatgagacaataaccctgataaatgcttcaataatattgaaaaaggaagagtatgagtattcaacatttccgtgtcgcccttattcccttttttgcggcattttgccttcctgtttttgctcacccagaaacgctggtgaaagtaaaagatgctgaagatcagttgggtgcacgagtgggttacatcgaactggatctcaacagcggtaagatccttgagagttttcgccccgaagaacgttttccaatgatgagcacttttaaagttctgctatgtggcgcggtattatcccgtattgacgccgggcaagagcaactcggtcgccgcatacactattctcagaatgacttggttgagtactcaccagtcacagaaaagcatcttacggatggcatgacagtaagagaattatgcagtgctgccataaccatgagtgataacactgcggccaacttacttctgacaacgatcggaggaccgaaggagctaaccgcttttttgcacaacatgggggatcatgtaactcgccttgatcgttgggaaccggagctgaatgaagccataccaaacgacgagcgtgacaccacgatgcctgcagcaatggcaacaacgttgcgcaaactattaactggcgaactacttactctagcttcccggcaacaattaatagactggatggaggcggataaagttgcaggaccacttctgcgctcggcccttccggctggctggtttattgctgataaatctggagccggtgagcgtgggtctcgcggtatcattgcagcactggggccagatggtaagccctcccgtatcgtagttatctacacgacggggagtcaggcaactatggatgaacgaaatagacagatcgctgagataggtgcctcactgattaagcattggtaactgtcagaccaagtttactcatatatactttagattgatttaaaacttcatttttaatttaaaaggatctaggtgaagatcctttttgataatctcatgaccaaaatcccttaacgtgagttttcgttccactgagcgtcagaccccgtagaaaagatcaaaggatcttcttgagatcctttttttctgcgcgtaatctgctgcttgcaaacaaaaaaaccaccgctaccagcggtggtttgtttgccggatcaagagctaccaactctttttccgaaggtaactggcttcagcagagcgcagataccaaatactgtccttctagtgtagccgtagttaggccaccacttcaagaactctgtagcaccgcctacatacctcgctctgctaatcctgttaccagtggctgctgccagtggcgataagtcgtgtcttaccgggttggactcaagacgatagttaccggataaggcgcagcggtcgggctgaacggggggttcgtgcacacagcccagcttggagcgaacgacctacaccgaactgagatacctacagcgtgagctatgagaaagcgccacgcttcccgaagggagaaaggcggacaggtatccggtaagcggcagggtcggaacaggagagcgcacgagggagcttccagggggaaacgcctggtatctttatagtcctgtcgggtttcgccacctctgacttgagcgtcgatttttgtgatgctcgtcaggggggcggagcctatggaaaaacgccagcaacgcggcctttttacggttcctggccttttgctggccttttgctcacatgttctttcctgcgttatcccctgattctgtggataaccgtattaccgcctttgagtgagctgataccgctcgccgcagccgaacgaccgagcgcagcgagtcagtgagcgaggaagcggaagagcgcctgatgcggtattttctccttacgcatctgtgcggtatttcacaccgcatatatggtgcactctcagtacaatctgctctgatgccgcatagttaagccagtatacactccgctatcgctacgtgactgggtcatggctgcgccccgacacccgccaacacccgctgacgcgccctgacgggcttgtctgctcccggcatccgcttacagacaagctgtgaccgtctccgggagctgcatgtgtcagaggttttcaccgtcatcaccgaaacgcgcgaggcagctgcggtaaagctcatcagcgtggtcgtgaagcgattcacagatgtctgcctgttcatccgcgtccagctcgttgagtttctccagaagcgttaatgtctggcttctgataaagcgggccatgttaagggcggttttttcctgtttggtcactgatgcctccgtgtaagggggatttctgttcatgggggtaatgataccgatgaaacgagagaggatgctcacgatacgggttactgatgatgaacatgcccggttactggaacgttgtgagggtaaacaactggcggtatggatgcggcgggaccagagaaaaatcactcagggtcaatgccagcgcttcgttaatacagatgtaggtgttccacagggtagccagcagcatcctgcgatgcagatccggaacataatggtgcagggcgctgacttccgcgtttccagactttacgaaacacggaaaccgaagaccattcatgttgttgctcaggtcgcagacgttttgcagcagcagtcgcttcacgttcgctcgcgtatcggtgattcattctgctaaccagtaaggcaaccccgccagcctagccgggtcctcaacgacaggagcacgatcatgcgcacccgtggggccgccatgccggcgataatggcctgcttctcgccgaaacgtttggtggcgggaccagtgacgaaggcttgagcgagggcgtgcaagattccgaataccgcaagcgacaggccgatcatcgtcgcgctccagcgaaagcggtcctcgccgaaaatgacccagagcgctgccggcacctgtcctacgagttgcatgataaagaagacagtcataagtgcggcgacgatagtcatgccccgcgcccaccggaaggagctgactgggttgaaggctctcaagggcatcggtcgagatcccggtgcctaatgagtgagctaacttacattaattgcgttgcgctcactgcccgctttccagtcgggaaacctgtcgtgccagctgcattaatgaatcggccaacgcgcggggagaggcggtttgcgtattgggcgccagggtggtttttcttttcaccagtgagacgggcaacagctgattgcccttcaccgcctggccctgagagagttgcagcaagcggtccacgctggtttgccccagcaggcgaaaatcctgtttgatggtggttaacggcgggatataacatgagctgtcttcggtatcgtcgtatcccactaccgagatatccgcaccaacgcgcagcccggactcggtaatggcgcgcattgcgcccagcgccatctgatcgttggcaaccagcatcgcagtgggaacgatgccctcattcagcatttgcatggtttgttgaaaaccggacatggcactccagtcgccttcccgttccgctatcggctgaatttgattgcgagtgagatatttatgccagccagccagacgcagacgcgccgagacagaacttaatgggcccgctaacagcgcgatttgctggtgacccaatgcgaccagatgctccacgcccagtcgcgtaccgtcttcatgggagaaaataatactgttgatgggtgtctggtcagagacatcaagaaataacgccggaacattagtgcaggcagcttccacagcaatggcatcctggtcatccagcggatagttaatgatcagcccactgacgcgttgcgcgagaagattgtgcaccgccgctttacaggcttcgacgccgcttcgttctaccatcgacaccaccacgctggcacccagttgatcggcgcgagatttaatcgccgcgacaatttgcgacggcgcgtgcagggccagactggaggtggcaacgccaatcagcaacgactgtttgcccgccagttgttgtgccacgcggttgggaatgtaattcagctccgccatcgccgcttccactttttcccgcgttttcgcagaaacgtggctggcctggttcaccacgcgggaaacggtctgataagagacaccggcatactctgcgacatcgtataacgttactggtttcacattcaccaccctgaattgactctcttccgggcgctatcatgccataccgcgaaaggttttgcgccattcgatggtgtccgggatctcgacgctctcccttatgcgactcctgcattaggaagcagcccagtagtaggttgaggccgttgagcaccgccgccgcaaggaatggtgcatgcaaggagatggcgcccaacagtcccccggccacggggcctgccaccatacccacgccgaaacaagcgctcatgagcccgaagtggcgagcccgatcttccccatcggtgatgtcggcgatataggcgccagcaaccgcacctgtggcgccggtgatgccggccacgatgcgtccggcgtagaggatcgagatctcgatcccgcgaaattaatacgactcactataggggaattgtgagcggataacaattcccctctagaaataattttgtttaactttaagaaggagatatacatggcacatattgttatggttgatgcctataaaccgaccaaaggtggtggtggcagcgttagcaaaggtgaagaactgtttaccggtgttgttccgattctggttgaactggatggtgatgttaatggccacaaattttcagttagcggtgaaggtgagggtgatgcaacctatggtaaactgaccctgaaatttatctgcaccaccggcaaactgccggttccgtggccgaccctggttaccaccctgacctatggtgttcagtgttttagccgttatccggatcatatgaaacagcacgattttttcaaaagcgcaatgccggaaggttatgttcaagaacgtaccatctttttcaaagacgacggcaactataaaacccgtgccgaagttaaatttgaaggtgataccctggtgaatcgcattgaactgaaaggcatcgattttaaagaagatggcaatatcctgggccacaaactggaatataattataatagccacaacgtgtacatcatggccgacaaacagaaaaatggcatcaaagtgaacttcaaaatccgccacaatattgaagatggctcagttcagctggcagatcattatcagcagaataccccgatcggtgatggtccggttctgctgccggataatcattatctgagcacccagagcgcactgagcaaagatccgaatgaaaaacgtgatcacatggtgctgctggaatttgttaccgcagcaggtattaccctgggtatggatgaactgtataaacatcatcaccaccatcattaagatccggctgctaacaaagcccgaaaggaa